European Patent Specification EP 3 157 542 B1, published December 25, 2024. Title: METHODS TO TREAT INFLAMMATION OF THE LUNG. Applicant: Rutgers, the State University of New Jersey. The sequence listing filed with the application follows.

SEQUENCE LISTING (2 sequences)

SEQ ID NO: 1 - protein, 1055 aa, Aggregatibacter actinomycetemcomitans
MATTSLLNTKQQAAQFANSVADRAKENIDAAKEQLQKALDKLGKTGKKLTLYIKNYKKGNGLTALIKAAQKLGIEVYHEGKDGPALTNGILNTGKKLLGLTERGLTLFAPELDKWIQGNKHLSNSVGSTGNLTKAIDKVQSVLGTLQAFLNTAFSGMDLDALIKARQNGKNVTDVQLAKASLNLINELIGTISSITNNVDTFSKQLNKLGEALGQVKHFGSFGDKLKNLPKLGNLGKGLGALSGVLSAISAALLLANKDADTATKAAAAAELTNKVLGNIGKAITQYLIAQRAAAGLSTTGPVAGLIASVVSLAISPLSFLGIAKQFDRARMLEEYSKRFKKFGYNGDSLLGQFYKNTGIADAAITTINTVLSAIAAGVGAASAGSLVGAPIGLLVSAITSLISGILDASKQAVFEHIANQLADKIKAWENKYGKNYFENGYDARHSAFLEDSLKLFNELREKYKTENILSITQQGWDQRIGELAGITRNGDRIQSGKAYVDYLKKGEELAKHSDKFTKQILDPIKGNIDLSGIKGSTTLTFLNPLLTAGKEERKTRQSGKYEFITELKVKGRTDWKVKGVPNSNGVYDFSNLIQHAVTRDNKVLEARLIANLGAKDDYVFVGSGSTIVNAGDGYDVVDYSKGRTGALTIDGRNATKAGQYKVERDLSGTQVLQETVSKQETKRGKVTDLLEYRNYKLDYYYTNKGFKAHDELNSVEEIIGSTLRDKFYGSKFNDVFHGHDGDDLIYGYDGDDRLYGDNGNDEIHGGQGNDKLYGGAGNDRLFGEYGNNYLDGGEGDDHLEGGNGSDILRGGSGNDKLFGNQGDDLLDGGEGDDQLAGGEGNDIYVYRKEYGHHTITEHSGDKDKLSLANINLKDVSFERNGNDLLLKTNNRTAVTFKGWFSKPNSSAGLDEYQRKLLEYAPEKDRARLKRQFELQRGKVDKSLNNKVEEIIGKDGERITSQDIDNLFDKSGNKKTISPQELAGLIKNKGKSSSLMSSSRSSSMLTQKSGLSNDISRIISATSGFGSSGKALSASPLQTNNNFNSYANSLATTAA

SEQ ID NO: 2 - DNA, 3168 bp, Aggregatibacter actinomycetemcomitans
atggcaactacttcactgctaaatacaaaacagcaagctgcacagtttgcaaattcagttgcagatagagctaaggaaaatattgatgctgcaaaagaacaattgcaaaaggcgttagataaattagggaagacaggtaagaaattaactttatatatccctaagaattacaaaaaaggaaatggtcttactgcgcttataaaagcagcacagaagttagggattgaagtatatcatgaagggaaagacggcccggcattaactaatggtattttaaatactgggaaaaaattacttggtcttaccgaacgaggtttaactttatttgctccggaattagataaatggattcaaggtaataaacatttaagtaattctgtgggtagtactggaaatttgacaaaagcgatagataaggttcagagtgttcttggtacgttacaagcgtttttgaacaccgcattttcgggcatggatttagatgccttaattaaagcccgtcaaaatggtaaaaatgtaacagatgtacagctagcaaaagccagtcttaacctgattaatgaattgattggtactatttctagcattacaaataatgtagatactttttctaaacaacttaataagttaggtgaagcactaggacaagtaaaacattttggtagttttggagataaattaaagaatttacctaagttaggtaatcttggaaaaggtttaggtgcattatccggtgtattgtcggctatatcagcggctctattacttgcaaataaagatgctgatactgcaacgaaagcagcggctgcagctgaattgacaaataaagtgctaggtaacatcggtaaagcgatcacacaatacttgattgctcaacgtgctgcagcggggctttctactacgggacctgtcgcagggttaattgcctctgtggtcagcttggcaatcagccctttgtctttcctaggtattgcgaaacaatttgatcgtgcgagaatgcttgaggaatactcgaaacgctttaagaaatttggttataacggcgatagtttacttggtcaattctacaaaaatacagggatcgcagatgctgcgattacaacgattaacactgtattaagtgctattgcagcaggggttggtgcagcctccgccggttctttagttggtgcgccaatcggtttgttagtgagtgcgattaccagcttaatttcaggaattcttgatgcttctaaacaagccgtttttgaacatatcgcgaatcagctcgccgataaaattaaagcatgggagaataagtacggtaagaattactttgaaaatggctatgatgcccgtcattccgccttcttggaagattcactaaaattatttaatgagttacgtgaaaaatataaaaccgaaaatatattatctatcactcaacaaggttgggatcagcgcattggtgaattagcaggtatcactcgtaatggagatcgtattcaaagtggtaaagcttatgtggattatttgaaaaagggtgaggagcttgcaaagcatagcgataaattcactaaacagattttagatccaatcaaaggtaatattgatctttcgggtataaaaggttctaccactctaacttttttaaatccgttgttaaccgcaggtaaggaagaacggaaaacacgtcagtcaggtaaatatgaatttattactgaattaaaagtaaaaggacgtaccgattggaaggtaaaaggtgttcctaattctaatggtgtatatgatttttctaacttaattcaacatgccgttacacgtgataataaagttctagaagcaagattaattgctaatttgggtgctaaagatgattatgtttttgtcggatccggttcaacaatagttaatgctggagacggttatgatgtggtggactatagtaaaggtcgcaccggtgcattaacaatcgacggtcgtaatgctactaaagccggacaatataaggttgaaagagatcttagcggtactcaagtcttgcaggaaaccgtatcaaagcaagaaactaaacgagggaaggttaccgatctacttgaatatcgtaactataaattagattactattatacgaataagggctttaaagctcatgatgaattaaactcagtagaggaaattatcggcagcacactacgtgataaattttatggttctaaatttaatgatgttttccatggtcacgatggcgatgatttgatttatggttatgatggcgatgatcgtttgtatggcgataatgggaatgacgaaattcatggcggccaaggtaatgataagctctatggtggtgccggtaacgataggctctttggtgaatatggcaacaactatcttgacggtggagaaggcgacgaccacttagagggaggcaatggttccgatattctaagaggtggaagtggcaatgataagttgtttggaaaccaaggagatgatttacttgacggtggagaaggcgatgaccaacttgccggtggagaaggaaatgatatttatgtttaccgtaaagaatatgggcaccacactattacggaacatagcggtgataaagataaattatcattagcaaatatcaatctcaaagatgtgtcatttgagcgtaacggcaatgatctactattgaaaacaaataatagaacagcagtaacatttaaaggatggtttagtaaacctaattcatcggcaggattagatgagtatcaaagaaaacttcttgaatacgcacctgaaaaggatcgtgcacgacttaagagacaatttgagttacagcgaggtaaagtcgacaaatcactcaataataaagttgaagaaattatcggtaaagatggggagcggattacttcgcaagacattgataatctttttgataagagtgggaacaaaaagacaatttcacctcaagagcttgccggacttattaagaataaaggtaagtcaagtagccttatgtcttcttctcgttcgtcaagtatgcttacacaaaagtccggtttgtcaaatgatattagtcgtattatttcagcaaccagtggttttggttcatccggtaaagcgttatccgcttcgccattgcagaccaataataactttaactcttacgcaaattcgttagcaactactgcggcc